European Patent Specification EP 3 062 822 B1, published May 14, 2025. Title: Cell Transport. Applicant: Cupid Peptide Company Limited. The sequence listing filed with the application follows.

SEQUENCE LISTING (13 sequences)

SEQ ID NO: 1 - protein, 16 aa, Dictyostelium discoideum
RRVQIWFQNKRAKVKR

SEQ ID NO: 2 - protein, 15 aa, Dictyostelium discoideum
RSVQIWFQNRRAKAR

SEQ ID NO: 3 - DNA, 81 bp, Dictyostelium discoideum
gaatccatgcaccatcaccatcaccatagaagagttcaaatttggttccaaaataaacgtgctaaagtaaagagaatcgat

SEQ ID NO: 4 - DNA, 6 bp, Escherichia coli
gaatcc

SEQ ID NO: 5 - DNA, 18 bp, Dictyostelium discoideum
caccatcaccatcaccat

SEQ ID NO: 6 - DNA, 48 bp, Dictyostelium discoideum
agaagagttcaaatttggttccaaaataaacgtgctaaagtaaagaga

SEQ ID NO: 7 - DNA, 6 bp, Escherichia coli
atcgat

SEQ ID NO: 8 - protein, 16 aa, Drosophila melanogaster
RQIKIWFQNRRMKWKK

SEQ ID NO: 9 - protein, 20 aa, Dictyostelium discoideum [sequence omitted]

SEQ ID NO: 10 - protein, 167 aa, Homo sapiens
LDYRPVALLFHKMMFETIPMFSGGTCNPQFVVCQLKVKIYSSNSGPTRREDKFMYFEFPQPLPVCGDIKVEFFHKQNKMLKKDKMFHFWVNTFFIPGPEETSEKVENGSLCDQEIDSICSIERADNDKEYLVLTLTKNDLDKANKDKANRYFSPNFKVKLYFTKTVE

SEQ ID NO: 11 - protein, 44 aa, Drosophila melanogaster
HHHHHHRRVQIWFQNKRAKVKRIDTTYADFIASGRTGRRNAIHD

SEQ ID NO: 12 - protein, 191 aa, Homo sapiens
HHHHHHRRVQIWFQNKRAKVKRIDLDYRPVALLFHKMMFETIPMFSGGTCNPQFVVCQLKVKIYSSNSGPTRREDKFMYFEFPQPLPVCGDIKVEFFHKQNKMLKKDKMFHFWVNTFFIPGPEETSEKVENGSLCDQEIDSICSIERADNDKEYLVLTLTKNDLDKANKDKANRYFSPNFKVKLYFTKTVE

SEQ ID NO: 13 - protein, 254 aa, Aequorea victoria
MRRVQIWFQNKRAKVKRSKGEELFTGVVPILVELDGDVNGHKFSVSGEGEGDATYGKLTLKFICTTGKLPVPWPTLVTTFSYGVQCFSRYPDHMKQHDFFKSAMPEGYVQERTIFFKDDGNYKTRAEVKFEGDTLVNRIELKGIDFKEDGNILGHKLEYNYNSHNVYIMADKQKNGIKVNFKIRHNIEDGSVQLADHYQQNTPIGDGPVLLPDNHYLSTQSALSKDPNEKRDHMVLLEFVTAAGITHGMDELYK